European Patent Specification EP 3 549 599 B1, published September 6, 2023. Title: Antibodies. Applicant: UCB Biopharma Sprl. The sequence listing filed with the application follows.

SEQUENCE LISTING (39 sequences)

SEQ ID NO: 1 - protein, 11 aa, Artificial Sequence
  CA019_969 Ab sequences CDR-L1
LASEDIYDNLA

SEQ ID NO: 2 - protein, 7 aa, Artificial Sequence
  CA019_969 Ab sequences CDRL2
YASSLQD

SEQ ID NO: 3 - protein, 9 aa, Artificial Sequence
  CA019_969 Ab sequences CDR-L3
LQDSEYPWT

SEQ ID NO: 4 - protein, 12 aa, Artificial Sequence
  CA019_969 Ab sequences CDR-H1
GFSLTTYGMGVG

SEQ ID NO: 5 - protein, 16 aa, Artificial Sequence
  CA019_969 Ab sequences CDR-H2
NIWWDDDKYYNPSLKN

SEQ ID NO: 6 - protein, 16 aa, Artificial Sequence
  CA019_969 Ab sequences CDR-H3
IGPIKYPTAPYRYFDF

SEQ ID NO: 7 - protein, 107 aa, Artificial Sequence
  Rat Ab 969 VL region
DIQMTQSPASLSASLGETVSIECLASEDIYDNLAWYQKKPGKSPHLLIYYASSLQDGVPSRFSGSGSGTQYSLKINSLESEDAATYFCLQDSEYPWTFGGGTKLELK

SEQ ID NO: 8 - DNA, 321 bp, Artificial Sequence
  Rat Ab 969 VL region
gacatccagatgacacagtctccagcttccctgtctgcatctctgggagaaactgtctccatcgaatgtctagcaagtgaggacatttacgataatttagcgtggtaccagaagaagccaggaaaatctcctcacctcctcatctattatgcaagtagcttgcaagatggggtcccatcacggttcagtggcagtggatctggcacacagtattctctcaaaatcaacagcctggaatctgaagatgctgcgacttatttctgtctacaggattctgagtatccgtggacgttcggtggaggcaccaagctggaattgaaa

SEQ ID NO: 9 - protein, 127 aa, Artificial Sequence
  Rat Ab 969 VL region with signal sequence underlined and italicised
MGVPTQLLVLLLLWITDAICDIQMTQSPASLSASLGETVSIECLASEDIYDNLAWYQKKPGKSPHLLIYYASSLQDGVPSRFSGSGSGTQYSLKINSLESEDAATYFCLQDSEYPWTFGGGTKLELK

SEQ ID NO: 10 - DNA, 381 bp, Artificial Sequence
  Rat Ab 969 VL region with signal sequence underlined and italicised
atgggtgtccccactcagctcttggtgttgttgctgctgtggattacagatgccatatgtgacatccagatgacacagtctccagcttccctgtctgcatctctgggagaaactgtctccatcgaatgtctagcaagtgaggacatttacgataatttagcgtggtaccagaagaagccaggaaaatctcctcacctcctcatctattatgcaagtagcttgcaagatggggtcccatcacggttcagtggcagtggatctggcacacagtattctctcaaaatcaacagcctggaatctgaagatgctgcgacttatttctgtctacaggattctgagtatccgtggacgttcggtggaggcaccaagctggaattgaaa

SEQ ID NO: 11 - protein, 125 aa, Artificial Sequence
  Rat Ab 969 VH region
QVTLKESGPGILQPSQTLSLTCTFSGFSLTTYGMGVGWIRQPSGKGLEWLANIWWDDDKYYNPSLKNRLTISKDTSNNQAFLKLTNVHTSDSATYYCARIGPIKYPTAPYRYFDFWGPGTMVTVS

SEQ ID NO: 12 - DNA, 375 bp, Artificial Sequence
  Rat Ab 969 VH region
caggttactctgaaagagtctggccctgggatattgcagccctcccagaccctcagtctgacttgcactttctctgggttttcactgaccacttatggtatgggtgtgggctggattcgtcagccttcagggaagggtctggagtggctggcaaacatttggtgggatgatgataagtattacaatccatctctgaaaaaccggctcacaatctccaaggacacctccaacaaccaagcattcctcaagctcaccaatgtacacacttcagattctgccacatactactgtgctcggatagggccgattaaatacccgacggccccctaccggtactttgacttctggggcccaggaaccatggtcaccgtctcg

SEQ ID NO: 13 - protein, 144 aa, Artificial Sequence
  Rat Ab 969 VH region with signal sequence underlined and italicised
MDRLTSSFLLLIVPAYVLSQVTLKESGPGILQPSQTLSLTCTFSGFSLTTYGMGVGWIRQPSGKGLEWLANIWWDDDKYYNPSLKNRLTISKDTSNNQAFLKLTNVHTSDSATYYCARIGPIKYPTAPYRYFDFWGPGTMVTVS

SEQ ID NO: 14 - DNA, 432 bp, Artificial Sequence
  Rat Ab 969 VH region with signal sequence underlined and italicised
atggacaggcttacttcctcattcctactgctgattgtccctgcatatgtcctgtctcaggttactctgaaagagtctggccctgggatattgcagccctcccagaccctcagtctgacttgcactttctctgggttttcactgaccacttatggtatgggtgtgggctggattcgtcagccttcagggaagggtctggagtggctggcaaacatttggtgggatgatgataagtattacaatccatctctgaaaaaccggctcacaatctccaaggacacctccaacaaccaagcattcctcaagctcaccaatgtacacacttcagattctgccacatactactgtgctcggatagggccgattaaatacccgacggccccctaccggtactttgacttctggggcccaggaaccatggtcaccgtctcg

SEQ ID NO: 15 - protein, 107 aa, Artificial Sequence
  969 gL7 V-region
DIQMTQSPSSLSASVGDRVTITCLASEDIYDNLAWYQQKPGKAPKLLIYYASSLQDGVPSRFSGSGSGTDYTLTISSLQPEDFATYYCLQDSEYPWTFGGGTKVEIK

SEQ ID NO: 16 - DNA, 321 bp, Artificial Sequence
  969 gL7 V-region
gacatacagatgactcagtcaccctcaagcctgagtgccagtgtgggagacagggtgacaatcacctgtctggcctccgaggatatctacgataacctggcatggtatcagcagaaacctggaaaggctcccaagctcctgatttattatgcctcctctctccaagacggcgttccatctcggttcagcggaagcggctccgggacggattacacactgacaattagctctctgcaaccggaggattttgctacttactactgcctgcaagactccgaatacccatggaccttcggtggtggcaccaaagtggaaatcaag

SEQ ID NO: 17 - protein, 127 aa, Artificial Sequence
  969 gL7 V-region with signal sequence underlined and italicized
MSVPTQVLGLLLLWLTDARCDIQMTQSPSSLSASVGDRVTITCLASEDIYDNLAWYQQKPGKAPKLLIYYASSLQDGVPSRFSGSGSGTDYTLTISSLQPEDFATYYCLQDSEYPWTFGGGTKVEIK

SEQ ID NO: 18 - DNA, 381 bp, Artificial Sequence
  969 gL7 V-region with signal sequence underlined and italicized
atgagcgtgcctactcaagtcttggggctgctcttgctttggcttaccgacgcaagatgcgacatacagatgactcagtcaccctcaagcctgagtgccagtgtgggagacagggtgacaatcacctgtctggcctccgaggatatctacgataacctggcatggtatcagcagaaacctggaaaggctcccaagctcctgatttattatgcctcctctctccaagacggcgttccatctcggttcagcggaagcggctccgggacggattacacactgacaattagctctctgcaaccggaggattttgctacttactactgcctgcaagactccgaatacccatggaccttcggtggtggcaccaaagtggaaatcaag

SEQ ID NO: 19 - protein, 214 aa, Artificial Sequence
  969 gL7 light chain (V + constant)
DIQMTQSPSSLSASVGDRVTITCLASEDIYDNLAWYQQKPGKAPKLLIYYASSLQDGVPSRFSGSGSGTDYTLTISSLQPEDFATYYCLQDSEYPWTFGGGTKVEIKRTVAAPSVFIFPPSDEQLKSGTASVVCLLNNFYPREAKVQWKVDNALQSGNSQESVTEQDSKDSTYSLSSTLTLSKADYEKHKVYACEVTHQGLSSPVTKSFNRGEC

SEQ ID NO: 20 - DNA, 642 bp, Artificial Sequence
  969 gL7 light chain (V + constant)
gacatacagatgactcagtcaccctcaagcctgagtgccagtgtgggagacagggtgacaatcacctgtctggcctccgaggatatctacgataacctggcatggtatcagcagaaacctggaaaggctcccaagctcctgatttattatgcctcctctctccaagacggcgttccatctcggttcagcggaagcggctccgggacggattacacactgacaattagctctctgcaaccggaggattttgctacttactactgcctgcaagactccgaatacccatggaccttcggtggtggcaccaaagtggaaatcaagcgtacggtagcggccccatctgtcttcatcttcccgccatctgatgagcagttgaaatctggaactgcctctgttgtgtgcctgctgaataacttctatcccagagaggccaaagtacagtggaaggtggataacgccctccaatcgggtaactcccaggagagtgtcacagagcaggacagcaaggacagcacctacagcctcagcagcaccctgacgctgagcaaagcagactacgagaaacacaaagtctacgcctgcgaagtcacccatcagggcctgagctcgcccgtcacaaagagcttcaacaggggagagtgt

SEQ ID NO: 21 - protein, 234 aa, Artificial Sequence
  969 gL7 light chain (V + constant) with signal sequence underlined and italicized
MSVPTQVLGLLLLWLTDARCDIQMTQSPSSLSASVGDRVTITCLASEDIYDNLAWYQQKPGKAPKLLIYYASSLQDGVPSRFSGSGSGTDYTLTISSLQPEDFATYYCLQDSEYPWTFGGGTKVEIKRTVAAPSVFIFPPSDEQLKSGTASVVCLLNNFYPREAKVQWKVDNALQSGNSQESVTEQDSKDSTYSLSSTLTLSKADYEKHKVYACEVTHQGLSSPVTKSFNRGEC

SEQ ID NO: 22 - DNA, 702 bp, Artificial Sequence
  969 gL7 light chain (V + constant) with signal sequence underlined and italicized
atgagcgtgcctactcaagtcttggggctgctcttgctttggcttaccgacgcaagatgcgacatacagatgactcagtcaccctcaagcctgagtgccagtgtgggagacagggtgacaatcacctgtctggcctccgaggatatctacgataacctggcatggtatcagcagaaacctggaaaggctcccaagctcctgatttattatgcctcctctctccaagacggcgttccatctcggttcagcggaagcggctccgggacggattacacactgacaattagctctctgcaaccggaggattttgctacttactactgcctgcaagactccgaatacccatggaccttcggtggtggcaccaaagtggaaatcaagcgtacggtagcggccccatctgtcttcatcttcccgccatctgatgagcagttgaaatctggaactgcctctgttgtgtgcctgctgaataacttctatcccagagaggccaaagtacagtggaaggtggataacgccctccaatcgggtaactcccaggagagtgtcacagagcaggacagcaaggacagcacctacagcctcagcagcaccctgacgctgagcaaagcagactacgagaaacacaaagtctacgcctgcgaagtcacccatcagggcctgagctcgcccgtcacaaagagcttcaacaggggagagtgt

SEQ ID NO: 23 - protein, 125 aa, Artificial Sequence
  969 gH2 V-region
EVTLKESGPALVKPTQTLTLTCTFSGFSLTTYGMGVGWIRQPPGKALEWLANIWWDDDKYYNPSLKNRLTISKDTSKNQVVLTMTNMDPVDTATYYCARIGPIKYPTAPYRYFDFWGQGTMVTVS

SEQ ID NO: 24 - DNA, 375 bp, Artificial Sequence
  969 gH2 V-region
gaagtgacactcaaggagtctggacccgctctggtgaaaccaacccaaacactcactttgacatgtacttttagtggcttctcattgactacctatggaatgggcgtgggatggatcagacagccacctggcaaggctctggaatggctggccaacatctggtgggatgacgacaagtactataacccgtccctgaaaaaccggctgaccattagcaaggatacttctaaaaatcaagtggtgctgaccatgacaaatatggatcccgttgacaccgcaacctactactgcgcccgcattggtcccataaagtaccctacggcaccttaccgatatttcgacttttggggccaagggacaatggttactgtctcg

SEQ ID NO: 25 - protein, 144 aa, Artificial Sequence
  969 gH2 V-region with signal sequence underlined and italicized
MEWSWVFLFFLSVTTGVHSEVTLKESGPALVKPTQTLTLTCTFSGFSLTTYGMGVGWIRQPPGKALEWLANIWWDDDKYYNPSLKNRLTISKDTSKNQVVLTMTNMDPVDTATYYCARIGPIKYPTAPYRYFDFWGQGTMVTVS

SEQ ID NO: 26 - DNA, 432 bp, Artificial Sequence
  969 gH2 V-region with signal sequence underlined and italicized
atggagtggtcctgggtgtttctgttcttcctgagtgtgaccaccggggtccactccgaagtgacactcaaggagtctggacccgctctggtgaaaccaacccaaacactcactttgacatgtacttttagtggcttctcattgactacctatggaatgggcgtgggatggatcagacagccacctggcaaggctctggaatggctggccaacatctggtgggatgacgacaagtactataacccgtccctgaaaaaccggctgaccattagcaaggatacttctaaaaatcaagtggtgctgaccatgacaaatatggatcccgttgacaccgcaacctactactgcgcccgcattggtcccataaagtaccctacggcaccttaccgatatttcgacttttggggccaagggacaatggttactgtctcg

SEQ ID NO: 27 - protein, 453 aa, Artificial Sequence
  969 gH2 heavy chain (V + constant - hu IgG4P)
EVTLKESGPALVKPTQTLTLTCTFSGFSLTTYGMGVGWIRQPPGKALEWLANIWWDDDKYYNPSLKNRLTISKDTSKNQVVLTMTNMDPVDTATYYCARIGPIKYPTAPYRYFDFWGQGTMVTVSSASTKGPSVFPLAPCSRSTSESTAALGCLVKDYFPEPVTVSWNSGALTSGVHTFPAVLQSSGLYSLSSVVTVPSSSLGTKTYTCNVDHKPSNTKVDKRVESKYGPPCPPCPAPEFLGGPSVFLFPPKPKDTLMISRTPEVTCVVVDVSQEDPEVQFNWYVDGVEVHNAKTKPREEQFNSTYRVVSVLTVLHQDWLNGKEYKCKVSNKGLPSSIEKTISKAKGQPREPQVYTLPPSQEEMTKNQVSLTCLVKGFYPSDIAVEWESNGQPENNYKTTPPVLDSDGSFFLYSRLTVDKSRWQEGNVFSCSVMHEALHNHYTQKSLSLSLGK

SEQ ID NO: 28 - DNA, 1966 bp, Artificial Sequence
  969 gH2 heavy chain (V + constant - hu IgG4P, exons underlined)
gaagtgacactcaaggagtctggacccgctctggtgaaaccaacccaaacactcactttgacatgtacttttagtggcttctcattgactacctatggaatgggcgtgggatggatcagacagccacctggcaaggctctggaatggctggccaacatctggtgggatgacgacaagtactataacccgtccctgaaaaaccggctgaccattagcaaggatacttctaaaaatcaagtggtgctgaccatgacaaatatggatcccgttgacaccgcaacctactactgcgcccgcattggtcccataaagtaccctacggcaccttaccgatatttcgacttttggggccaagggacaatggttactgtctcgagcgcttctacaaagggcccatccgtcttccccctggcgccctgctccaggagcacctccgagagcacagccgccctgggctgcctggtcaaggactacttccccgaaccggtgacggtgtcgtggaactcaggcgccctgaccagcggcgtgcacaccttcccggctgtcctacagtcctcaggactctactccctcagcagcgtggtgaccgtgccctccagcagcttgggcacgaagacctacacctgcaacgtagatcacaagcccagcaacaccaaggtggacaagagagttggtgagaggccagcacagggagggagggtgtctgctggaagccaggctcagccctcctgcctggacgcaccccggctgtgcagccccagcccagggcagcaaggcatgccccatctgtctcctcacccggaggcctctgaccaccccactcatgcccagggagagggtcttctggatttttccaccaggctccgggcagccacaggctggatgcccctaccccaggccctgcgcatacaggggcaggtgctgcgctcagacctgccaagagccatatccgggaggaccctgcccctgacctaagcccaccccaaaggccaaactctccactccctcagctcagacaccttctctcctcccagatctgagtaactcccaatcttctctctgcagagtccaaatatggtcccccatgcccaccatgcccaggtaagccaacccaggcctcgccctccagctcaaggcgggacaggtgccctagagtagcctgcatccagggacaggccccagccgggtgctgacgcatccacctccatctcttcctcagcacctgagttcctggggggaccatcagtcttcctgttccccccaaaacccaaggacactctcatgatctcccggacccctgaggtcacgtgcgtggtggtggacgtgagccaggaagaccccgaggtccagttcaactggtacgtggatggcgtggaggtgcataatgccaagacaaagccgcgggaggagcagttcaacagcacgtaccgtgtggtcagcgtcctcaccgtcctgcaccaggactggctgaacggcaaggagtacaagtgcaaggtctccaacaaaggcctcccgtcctccatcgagaaaaccatctccaaagccaaaggtgggacccacggggtgcgagggccacatggacagaggtcagctcggcccaccctctgccctgggagtgaccgctgtgccaacctctgtccctacagggcagccccgagagccacaggtgtacaccctgcccccatcccaggaggagatgaccaagaaccaggtcagcctgacctgcctggtcaaaggcttctaccccagcgacatcgccgtggagtgggagagcaatgggcagccggagaacaactacaagaccacgcctcccgtgctggactccgacggctccttcttcctctacagcaggctaaccgtggacaagagcaggtggcaggaggggaatgtcttctcatgctccgtgatgcatgaggctctgcacaaccactacacacagaagagcctctccctgtctctgggtaaa

SEQ ID NO: 29 - protein, 472 aa, Artificial Sequence
  969 gH2 heavy chain (V + constant - hu IgG4P) with signal sequence underlined and italicised
MEWSWVFLFFLSVTTGVHSEVTLKESGPALVKPTQTLTLTCTFSGFSLTTYGMGVGWIRQPPGKALEWLANIWWDDDKYYNPSLKNRLTISKDTSKNQVVLTMTNMDPVDTATYYCARIGPIKYPTAPYRYFDFWGQGTMVTVSSASTKGPSVFPLAPCSRSTSESTAALGCLVKDYFPEPVTVSWNSGALTSGVHTFPAVLQSSGLYSLSSVVTVPSSSLGTKTYTCNVDHKPSNTKVDKRVESKYGPPCPPCPAPEFLGGPSVFLFPPKPKDTLMISRTPEVTCVVVDVSQEDPEVQFNWYVDGVEVHNAKTKPREEQFNSTYRVVSVLTVLHQDWLNGKEYKCKVSNKGLPSSIEKTISKAKGQPREPQVYTLPPSQEEMTKNQVSLTCLVKGFYPSDIAVEWESNGQPENNYKTTPPVLDSDGSFFLYSRLTVDKSRWQEGNVFSCSVMHEALHNHYTQKSLSLSLGK

SEQ ID NO: 30 - DNA, 2023 bp, Artificial Sequence
  969 gH2 heavy chain (V + constant - hu IgG4P, exons underlined) with signal sequence underlined and italicized
atggagtggtcctgggtgtttctgttcttcctgagtgtgaccaccggggtccactccgaagtgacactcaaggagtctggacccgctctggtgaaaccaacccaaacactcactttgacatgtacttttagtggcttctcattgactacctatggaatgggcgtgggatggatcagacagccacctggcaaggctctggaatggctggccaacatctggtgggatgacgacaagtactataacccgtccctgaaaaaccggctgaccattagcaaggatacttctaaaaatcaagtggtgctgaccatgacaaatatggatcccgttgacaccgcaacctactactgcgcccgcattggtcccataaagtaccctacggcaccttaccgatatttcgacttttggggccaagggacaatggttactgtctcgagcgcttctacaaagggcccatccgtcttccccctggcgccctgctccaggagcacctccgagagcacagccgccctgggctgcctggtcaaggactacttccccgaaccggtgacggtgtcgtggaactcaggcgccctgaccagcggcgtgcacaccttcccggctgtcctacagtcctcaggactctactccctcagcagcgtggtgaccgtgccctccagcagcttgggcacgaagacctacacctgcaacgtagatcacaagcccagcaacaccaaggtggacaagagagttggtgagaggccagcacagggagggagggtgtctgctggaagccaggctcagccctcctgcctggacgcaccccggctgtgcagccccagcccagggcagcaaggcatgccccatctgtctcctcacccggaggcctctgaccaccccactcatgcccagggagagggtcttctggatttttccaccaggctccgggcagccacaggctggatgcccctaccccaggccctgcgcatacaggggcaggtgctgcgctcagacctgccaagagccatatccgggaggaccctgcccctgacctaagcccaccccaaaggccaaactctccactccctcagctcagacaccttctctcctcccagatctgagtaactcccaatcttctctctgcagagtccaaatatggtcccccatgcccaccatgcccaggtaagccaacccaggcctcgccctccagctcaaggcgggacaggtgccctagagtagcctgcatccagggacaggccccagccgggtgctgacgcatccacctccatctcttcctcagcacctgagttcctggggggaccatcagtcttcctgttccccccaaaacccaaggacactctcatgatctcccggacccctgaggtcacgtgcgtggtggtggacgtgagccaggaagaccccgaggtccagttcaactggtacgtggatggcgtggaggtgcataatgccaagacaaagccgcgggaggagcagttcaacagcacgtaccgtgtggtcagcgtcctcaccgtcctgcaccaggactggctgaacggcaaggagtacaagtgcaaggtctccaacaaaggcctcccgtcctccatcgagaaaaccatctccaaagccaaaggtgggacccacggggtgcgagggccacatggacagaggtcagctcggcccaccctctgccctgggagtgaccgctgtgccaacctctgtccctacagggcagccccgagagccacaggtgtacaccctgcccccatcccaggaggagatgaccaagaaccaggtcagcctgacctgcctggtcaaaggcttctaccccagcgacatcgccgtggagtgggagagcaatgggcagccggagaacaactacaagaccacgcctcccgtgctggactccgacggctccttcttcctctacagcaggctaaccgtggacaagagcaggtggcaggaggggaatgtcttctcatgctccgtgatgcatgaggctctgcacaaccactacacacagaagagcctctccctgtctctgggtaaa

SEQ ID NO: 31 - protein, 107 aa, Artificial Sequence [sequence omitted]

SEQ ID NO: 32 - DNA, 321 bp, Artificial Sequence
  Human VK1 2-1-(1) O12 JK4 acceptor framework
gacatccagatgacccagtctccatcctccctgtctgcatctgtaggagacagagtcaccatcacttgccgggcaagtcagagcattagcagctatttaaattggtatcagcagaaaccagggaaagcccctaagctcctgatctatgctgcatccagtttgcaaagtggggtcccatcaaggttcagtggcagtggatctgggacagatttcactctcaccatcagcagtctgcaacctgaagattttgcaacttactactgtcaacagagttacagtacccctctcactttcggcggagggaccaaggtggagatcaaa

SEQ ID NO: 33 - protein, 114 aa, Artificial Sequence
  Human VH2 3-1 2-70 JH3 acceptor framework
QVTLKESGPALVKPTQTLTLTCTFSGFSLSTSGMRVSWIRQPPGKALEWLARIDWDDDKFYSTSLKTRLTISKDTSKNQVVLTMTNMDPVDTATYYCARIAFDIWGQGTMVTVS

SEQ ID NO: 34 - DNA, 342 bp, Artificial Sequence
  Human VH2 3-1 2-70 JH3 acceptor framework
caggtcaccttgaaggagtctggtcctgcgctggtgaaacccacacagaccctcacactgacctgcaccttctctgggttctcactcagcactagtggaatgcgtgtgagctggatccgtcagcccccagggaaggccctggagtggcttgcacgcattgattgggatgatgataaattctacagcacatctctgaagaccaggctcaccatctccaaggacacctccaaaaaccaggtggtccttacaatgaccaacatggaccctgtggacacagccacgtattactgtgcacggatagcttttgatatctggggccaagggacaatggtcaccgtctct

SEQ ID NO: 35 - protein, 972 aa, Artificial Sequence
  Amino acid sequence for CSF-1R
MGPGVLLLLLVATAWHGQGIPVIEPSVPELVVKPGATVTLRCVGNGSVEWDGPPSPHWTLYSDGSSSILSTNNATFQNTGTYRCTEPGDPLGGSAAIHLYVKDPARPWNVLAQEVVVFEDQDALLPCLLTDPVLEAGVSLVRVRGRPLMRHTNYSFSPWHGFTIHRAKFIQSQDYQCSALMGGRKVMSISIRLKVQKVIPGPPALTLVPAELVRIRGEAAQIVCSASSVDVNFDVFLQHNNTKLAIPQQSDFHNNRYQKVLTLNLDQVDFQHAGNYSCVASNVQGKHSTSMFFRVVESAYLNLSSEQNLIQEVTVGEGLNLKVMVEAYPGLQGFNWTYLGPFSDHQPEPKLANATTKDTYRHTFTLSLPRLKPSEAGRYSFLARNPGGWRALTFELTLRYPPEVSVIWTFINGSGTLLCAASGYPQPNVTWLQCSGHTDRCDEAQVLQVWDDPYPEVLSQEPFHKVTVQSLLTVETLEHNQTYECRAHNSVGSGSWAFIPISAGAHTHPPDEFLFTPVVVACMSIMALLLLLLLLLLYKYKQKPKYQVRWKIIESYEGNSYTFIDPTQLPYNEKWEFPRNNLQFGKTLGAGAFGKVVEATAFGLGKEDAVLKVAVKMLKSTAHADEKEALMSELKIMSHLGQHENIVNLLGACTHGGPVLVITEYCCYGDLLNFLRRKAEAMLGPSLSPGQDPEGGVDYKNIHLEKKYVRRDSGFSSQGVDTYVEMRPVSTSSNDSFSEQDLDKEDGRPLELRDLLHFSSQVAQGMAFLASKNCIHRDVAARNVLLTNGHVAKIGDFGLARDIMNDSNYIVKGNARLPVKWMAPESIFDCVYTVQSDVWSYGILLWEIFSLGLNPYPGILVNSKFYKLVKDGYQMAQPAFAPKNIYSIMQACWALEPTHRPTFQQICSFLQEQAQEDRRERDYTNLPSSSRSGGSGSSSSELEEESSSEHLTCCEQGDIAQPLLQPNNYQFC

SEQ ID NO: 36 - protein, 277 aa, Artificial Sequence
  Amino acid sequence for CSF-1R
IPVIEPSVPELVVKPGATVTLRCVGNGSVEWDGPPSPHWTLYSDGSSSILSTNNATFQNTGTYRCTEPGDPLGGSAAIHLYVKDPARPWNVLAQEVVVFEDQDALLPCLLTDPVLEAGVSLVRVRGRPLMRHTNYSFSPWHGFTIHRAKFIQSQDYQCSALMGGRKVMSISIRLKVQKVIPGPPALTLVPAELVRIRGEAAQIVCSASSVDVNFDVFLQHNNTKLAIPQQSDFHNNRYQKVLTLNLDQVDFQHAGNYSCVASNVQGKHSTSMFFRVV

SEQ ID NO: 37 - protein, 49 aa, Artificial Sequence
  Amino acid sequence for CSF-1R
MRHTNYSFSPWHGFTIHRAKFIQSQDYQCSALMGGRKVMSISIRLKVQK

SEQ ID NO: 38 - protein, 493 aa, Artificial Sequence
  Amino acid sequence for CSF-1R (SNP V32G, A245S, H247P, V279M, position underlined)
IPVIEPSVPELVVKPGATVTLRCVGNGSVEWDGPPSPHWTLYSDGSSSILSTNNATFQNTGTYRCTEPGDPLGGSAAIHLYVKDPARPWNVLAQEVVVFEDQDALLPCLLTDPVLEAGVSLVRVRGRPLMRHTNYSFSPWHGFTIHRAKFIQSQDYQCSALMGGRKVMSISIRLKVQKVIPGPPALTLVPAELVRIRGEAAQIVCSASSVDVNFDVFLQHNNTKLAIHQQSDFHNNRYQKVLTLNLDQVDFQHAGNYSCVASNVQGKHSTSMFFRVVESAYLNLSSEQNLIQEVTVGEGLNLKVMVEAYPGLQGFNWTYLGPFSDHQPEPKLANATTKDTYRHTFTLSLPRLKPSEAGRYSFLARNPGGWRALTFELTLRYPPEVSVIWTFINGSGTLLCAASGYPQPNVTWLQCSGHTDRCDEAQVLQVWDDPYPEVLSQEPFHKVTVQSLLTVETLEHNQTYECRAHNSVGSGSWAFIPISAGAHTHPPDE

SEQ ID NO: 39 - protein, 512 aa, Artificial Sequence
  sequence of human CSF-1R extracellular domain
MGPGVLLLLLVATAWHGQGIPVIEPSVPELVVKPGATVTLRCVGNGSVEWDGPPSPHWTLYSDGSSSILSTNNATFQNTGTYRCTEPGDPLGGSAAIHLYVKDPARPWNVLAQEVVVFEDQDALLPCLLTDPVLEAGVSLVRVRGRPLMRHTNYSFSPWHGFTIHRAKFIQSQDYQCSALMGGRKVMSISIRLKVQKVIPGPPALTLVPAELVRIRGEAAQIVCSASSVDVNFDVFLQHNNTKLAIPQQSDFHNNRYQKVLTLNLDQVDFQHAGNYSCVASNVQGKHSTSMFFRVVESAYLNLSSEQNLIQEVTVGEGLNLKVMVEAYPGLQGFNWTYLGPFSDHQPEPKLANATTKDTYRHTFTLSLPRLKPSEAGRYSFLARNPGGWRALTFELTLRYPPEVSVIWTFINGSGTLLCAASGYPQPNVTWLQCSGHTDRCDEAQVLQVWDDPYPEVLSQEPFHKVTVQSLLTVETLEHNQTYECRAHNSVGSGSWAFIPISAGAHTHPPDE